European Patent Application EP 4 803 531 A1, published September 9, 2026. Title: 炭素環式ヌクレオシド含有オリゴヌクレオチド. Applicant: リードファーマ株式会社. The sequence listing filed with the application follows.

SEQUENCE LISTING (14 sequences)

SEQ ID NO: 1 - DNA, 24 bp, synthetic construct
  source 1..24: mol_type = other DNA
ttctcaagagttacagcagatcca

SEQ ID NO: 2 - DNA, 25 bp, synthetic construct
  source 1..25: mol_type = other DNA
tggaagtccttaagagcaactaaca

SEQ ID NO: 3 - DNA, 20 bp, synthetic construct
  source 1..20: mol_type = other DNA
gcaccgtcaaggctgagaac

SEQ ID NO: 4 - DNA, 19 bp, synthetic construct
  source 1..19: mol_type = other DNA
tggtgaagacgccagtgga

SEQ ID NO: 5 - DNA, 24 bp, synthetic construct
  source 1..24: mol_type = other DNA
tcctcggtgagttcaatgactttc

SEQ ID NO: 6 - DNA, 23 bp, synthetic construct
  source 1..23: mol_type = other DNA
tggacctgctgtagcttgtagga

SEQ ID NO: 7 - DNA, 20 bp, synthetic construct
  source 1..20: mol_type = other DNA
tgtgtccgtcgtggatctga

SEQ ID NO: 8 - DNA, 21 bp, synthetic construct
  source 1..21: mol_type = other DNA
ttgctgttgaagtcgcaggag

SEQ ID NO: 9 - DNA, 20 bp, synthetic construct
  source 1..20: mol_type = other DNA
tcagttctgcacacctccag

SEQ ID NO: 10 - DNA, 20 bp, synthetic construct
  source 1..20: mol_type = other DNA
gggtaaggtgcggtaagtcc

SEQ ID NO: 11 - DNA, 19 bp, synthetic construct
  source 1..19: mol_type = other DNA
aagggaagggcacggttag

SEQ ID NO: 12 - DNA, 20 bp, synthetic construct
  source 1..20: mol_type = other DNA
gagtagaggcaggcatcgtc

SEQ ID NO: 13 - DNA, 20 bp, synthetic construct
  source 1..20: mol_type = other DNA
ctgctccaggaacagaggtg

SEQ ID NO: 14 - DNA, 20 bp, synthetic construct
  source 1..20: mol_type = other DNA
gtggcgtgcttcatgtaacc